European Patent Application EP 4 292 612 A1, published December 20, 2023. Title: Human monomeric CRP-specific neutralizing antibody and medicament and anti-inflammatory agent containing the same. Applicant: CANON MEDICAL SYSTEMS CORPORATION General Incorporated Association The Japan-Multinational Trial Organization. The sequence listing filed with the application follows.

SEQUENCE LISTING (59 sequences)

SEQ ID NO: 1 - protein, 224 aa, Homo sapiens
MEKLLCFLVLTSLSHAFGQTDMSRKAFVFPKESDTSYVSLKAPLTKPLKAFTVCLHFYTELSSTRGYSIFSYATKRQDNEILIFWSKDIGYSFTVGGSEILFEVPEVTVAPVHICTSWESASGIVEFWVDGKPRVRKSLKKGYTVGAEASIILGQEQDSFGGNFEGSQSLVGDIGNVNMWDFVLSPDEINTIYLGGPFSPNVLNWRALKYEVQGEVFTKPQLWP

SEQ ID NO: 2 - protein, 10 aa, Artificial Sequence
  Epitope
EILFEVPEVT

SEQ ID NO: 3 - DNA, 1410 bp, Artificial Sequence
  Nucleotide sequence of polynucleotide encoding the heavy chain of the antibody 3C
atggaatggagctgggtctttctcttcctcctgtcagtaactgcaggtgtccaatcccaggttcagctgcagcagtctggggctgagctggtgaggcctggggcttcagtgaaactgtcctgcaaggctttggactacacatttactgactatgaaatgcactgggtgaaacagacacctgtgcatggcctggaatggattggagctattcatccaggaagaggtggtactgcctacaatcagaagttcaagggcaaggccacactgactgcagacaaatcctccagcacagcctacatggagctcagcagcctgacatctgaggactctggtgtctattactgtacaagttaccacggtggctactggggccaaggcaccactctcacagtctcctcagccaaaacaacacccccatcagtctatccactggcccctgggtgtggagatacaactggttcctccgtgactctgggatgcctggtcaagggctacttccctgagtcagtgactgtgacttggaactctggatccctgtccagcagtgtgcacaccttcccagctctcctgcagtctggactctacactatgagcagctcagtgactgtcccctccagcacctggccaagtcagaccgtcacctgcagcgttgctcacccagccagcagcaccacggtggacaaaaaacttgagcccagcgggcccatttcaacaatcaacccctgtcctccatgcaaggagtgtcacaaatgcccagctcctaacctcgagggtggaccatccgtcttcatcttccctccaaatatcaaggatgtactcatgatccccctgacacccaaggtcacgtgtgtggtggtggatgtgagcgaggatgacccagacgtccagatcagctggtttgtgaacaacgtggaagtacacacagctcagacacaaacccatagagaggattacaacagtactatccgggtggtcagcaccctccccatccagcaccaggactggatgagtggcaaggagttcaaatgcaaggtcaacaacaaagacctcccatcacccatcgagagaaccatctcaaaaattaaagggctagtcagagctccacaagtatacatcttgccgccaccagcagagcagttgtccaggaaagatgtcagtctcacttgcctggtcgtgggcttcaaccctggagacatcagtgtggagtggaccagcaatgggcatacagaggagaactacaaggacaccgcaccagtcctggactctgacggttcttacttcatatatagcaagctcaatatgaaaacaagcaagtgggagaaaacagattccttctcatgcaacgtgagacacgagggtctgaaaaattactacctgaagaagaccatctcccactctcctggtaaataa

SEQ ID NO: 4 - protein, 469 aa, Artificial Sequence
  Amino acid sequence of the heavy chain of the antibody 3C
MEWSWVFLFLLSVTAGVQSQVQLQQSGAELVRPGASVKLSCKALDYTFTDYEMHWVKQTPVHGLEWIGAIHPGRGGTAYNQKFKGKATLTADKSSSTAYMELSSLTSEDSGVYYCTSYHGGYWGQGTTLTVSSAKTTPPSVYPLAPGCGDTTGSSVTLGCLVKGYFPESVTVTWNSGSLSSSVHTFPALLQSGLYTMSSSVTVPSSTWPSQTVTCSVAHPASSTTVDKKLEPSGPISTINPCPPCKECHKCPAPNLEGGPSVFIFPPNIKDVLMIPLTPKVTCVVVDVSEDDPDVQISWFVNNVEVHTAQTQTHREDYNSTIRVVSTLPIQHQDWMSGKEFKCKVNNKDLPSPIERTISKIKGLVRAPQVYILPPPAEQLSRKDVSLTCLVVGFNPGDISVEWTSNGHTEENYKDTAPVLDSDGSYFIYSKLNMKTSKWEKTDSFSCNVRHEGLKNYYLKKTISHSPGK

SEQ ID NO: 5 - protein, 5 aa, Artificial Sequence
  CDR1 of Heavy chain found in the antibody 3C
DYEMH

SEQ ID NO: 6 - protein, 17 aa, Artificial Sequence
  CDR2 of Heavy chain found in the antibody 3C
AIHPGRGGTAYNQKFKG

SEQ ID NO: 7 - protein, 5 aa, Artificial Sequence
  CDR3 of Heavy chain found in the antibody 3C
YHGGY

SEQ ID NO: 8 - DNA, 717 bp, Artificial Sequence
  Nucleotide sequence of polynucleotide encoding the light chain of the antibody 3C
atgaagttgcctgttaggctgttggtgctgatgttctggattcctgctgcgagcagtgatgttgtgatgacccaaactccactctccctgcctgtcagtcttggagatcaagcctccatctcttgcagatctagtcagagccttgtacacagtaatgaaaacacctatttactttggtatctgcagaagccaggccagtctccaaagctcctgatctacaaagtttccaaccgattttctggggtcccagacaggttcagtggcagtggatcagggacagatttcacactcaagatcagcagagtggaggctgaggatctgggagtttatttctgctctcaaactacacatgttccgtggacgttcggtggaggcaccaagctggaaatcaaacgggctgatgctgcaccaactgtatccatcttcccaccatccagtgagcagttaacatctggaggtgcctcagtcgtgtgcttcttgaacaacttctaccccaaagacatcaatgtcaagtggaagattgatggcagtgaacgacaaaatggcgtcctgaacagttggactgatcaggacagcaaagacagcacctacagcatgagcagcaccctcacgttgaccaaggacgagtatgaacgacataacagctatacctgtgaggccactcacaagacatcaacttcacccattgtcaagagcttcaacaggaatgagtgttag

SEQ ID NO: 9 - protein, 238 aa, Artificial Sequence
  Amino acid sequence of the light chain of the antibody 3C
MKLPVRLLVLMFWIPAASSDVVMTQTPLSLPVSLGDQASISCRSSQSLVHSNENTYLLWYLQKPGQSPKLLIYKVSNRFSGVPDRFSGSGSGTDFTLKISRVEAEDLGVYFCSQTTHVPWTFGGGTKLEIKRADAAPTVSIFPPSSEQLTSGGASVVCFLNNFYPKDINVKWKIDGSERQNGVLNSWTDQDSKDSTYSMSSTLTLTKDEYERHNSYTCEATHKTSTSPIVKSFNRNEC

SEQ ID NO: 10 - protein, 16 aa, Artificial Sequence
  CDR1 of light chain found in the antibody 3C
RSSQSLVHSNENTYLL

SEQ ID NO: 11 - protein, 7 aa, Artificial Sequence
  CDR2 of light chain found in the antibody 3C
KVSNRFS

SEQ ID NO: 12 - protein, 9 aa, Artificial Sequence
  CDR3 of light chain found in the antibody 3C
SQTTHVPWT

SEQ ID NO: 13 - protein, 11 aa, Artificial Sequence
  Partial peptide of human CRP
QTDMSRKAFVC

SEQ ID NO: 14 - protein, 11 aa, Artificial Sequence
  Partial peptide of human CR
FPKESDTSYVC

SEQ ID NO: 15 - protein, 11 aa, Artificial Sequence
  Partial peptide of human CRP
SLKAPLTKPLC

SEQ ID NO: 16 - protein, 11 aa, Artificial Sequence
  Partial peptide of human CRP
KAFTVCLHFYC

SEQ ID NO: 17 - protein, 11 aa, Artificial Sequence
  Partial peptide of human CRP
TELSSTRGYSC

SEQ ID NO: 18 - protein, 11 aa, Artificial Sequence
  Partial peptide of human CRP
IFSYATKRQDC

SEQ ID NO: 19 - protein, 11 aa, Artificial Sequence
  Partial peptide of human CRP
NEILIFWSKDC

SEQ ID NO: 20 - protein, 11 aa, Artificial Sequence
  Partial peptide of human CRP
IGYSFTVGGSC

SEQ ID NO: 21 - protein, 11 aa, Artificial Sequence
  Partial peptide of human CRP
EILFEVPEVTC

SEQ ID NO: 22 - protein, 11 aa, Artificial Sequence
  Partial peptide of human CRP
VAPVHICTSWC

SEQ ID NO: 23 - protein, 11 aa, Artificial Sequence
  Partial peptide of human CRP
ESASGIVEFWC

SEQ ID NO: 24 - protein, 11 aa, Artificial Sequence
  Partial peptide of human CRP
VDGKPRVRKSC

SEQ ID NO: 25 - protein, 11 aa, Artificial Sequence
  Partial peptide of human CRP
LKKGYTVGAEC

SEQ ID NO: 26 - protein, 11 aa, Artificial Sequence
  Partial peptide of human CRP
ASIILGQEQDC

SEQ ID NO: 27 - protein, 11 aa, Artificial Sequence
  Partial peptide of human CRP
SFGGNFEGSQC

SEQ ID NO: 28 - protein, 11 aa, Artificial Sequence
  Partial peptide of human CRP
SLVGDIGNVNC

SEQ ID NO: 29 - protein, 11 aa, Artificial Sequence
  Partial peptide of human CRP
MWDFVLSPDEC

SEQ ID NO: 30 - protein, 11 aa, Artificial Sequence
  Partial peptide of human CRP
INTIYLGGPFC

SEQ ID NO: 31 - protein, 11 aa, Artificial Sequence
  Partial peptide of human CRP
SPNVLNWRALC

SEQ ID NO: 32 - protein, 17 aa, Artificial Sequence
  Partial peptide of human CRP
KYEVQGEVFTKPQLWPC

SEQ ID NO: 33 - protein, 31 aa, Artificial Sequence
  Partial peptide of human CRP
QTDMSRKAFVFPKESDTSYVSLKAPLTKPLC

SEQ ID NO: 34 - protein, 31 aa, Artificial Sequence
  Partial peptide of human CRP
KAFTVCLHFYTELSSTRGYSIFSYATKRQDC

SEQ ID NO: 35 - protein, 31 aa, Artificial Sequence
  Partial peptide of human CRP
NEILIFWSKDIGYSFTVGGSEILFEVPEVTC

SEQ ID NO: 36 - protein, 31 aa, Artificial Sequence
  Partial peptide of human CRP
VAPVHICTSWESASGIVEFWVDGKPRVRKSC

SEQ ID NO: 37 - protein, 31 aa, Artificial Sequence
  Partial peptide of human CRP
LKKGYTVGAEASIILGQEQDSFGGNFEGSQC

SEQ ID NO: 38 - protein, 31 aa, Artificial Sequence
  Partial peptide of human CRP
SLVGDIGNVNMWDFVLSPDEINTIYLGGPFC

SEQ ID NO: 39 - protein, 27 aa, Artificial Sequence
  Partial peptide of human CRP
SPNVLNWRALKYEVQGEVFTKPQLWPC

SEQ ID NO: 40 - DNA, 1389 bp, Artificial Sequence
  Heavy chain of chimeric antibody
atgggctggacattggtctttctcttcctgttgagcgtcactgcaggggtccactcacaggtgcaactgcagcagagtggggccgaactggttagacccggcgcaagtgttaagctgtcttgcaaggctctggactacaccttcactgactatgagatgcattgggtgaaacagacacctgtgcatggtctggaatggatcggagcaatacacccaggtcgaggaggaaccgcctataaccagaagtttaagggaaaagccaccttgactgctgataagtcctcttcaacagcctatatggagctttccagccttacttccgaggacagtggggtttactattgtaccagttatcacggaggttactggggacaggggaccacactgacagttagcagtgcctctacgaaaggcccctccgtgtttcctttggctccatcttcaaagtccacctcaggcggcaccgctgccctcggatgtctggtgaaggactacttccctgagcccgttactgtgtcatggaatagcggggctctgacttccggggtccacacatttcccgctgtacttcagtccagtggcttgtacagcctgtcctctgtggtcaccgttccaagctctagcctgggtacacagacctatatctgcaacgtaaaccataaaccctctaacacgaaggtagacaagaaagtcgagcctaagtcctgcgataagacccacacctgtccaccctgtcccgcacccgagctcctgggtggccctagcgtattcctgtttccacccaaaccaaaagacacactgatgatttccaggacacccgaggtgacatgcgtggtcgtggacgtgtctcatgaggaccccgaagtgaagttcaactggtatgttgatggagtcgaagtgcacaatgccaaaacgaagccacgcgaagaacagtacaactccacatatcgggtcgtatccgtcctgactgtgctccatcaggattggctgaatggcaaggagtacaaatgcaaggtgtccaataaggccttgcctgcacccatcgagaaaactatctccaaagccaaaggccagcctcgtgaacctcaagtgtacaccctgcctccatctagggatgagctgaccaagaaccaggtgtcactgacttgccttgtgaaaggcttttaccctagcgatattgctgttgaatgggagtccaatggtcagccagagaacaattacaagacaacccctccagtcctggactctgatgggagcttctttctctactctaagctcaccgtggataagagccggtggcaacaaggcaatgtgttcagttgttctgtgatgcatgaagccctccacaaccactatactcagaagtcactgagtcttagccccggtaaa

SEQ ID NO: 41 - protein, 463 aa, Artificial Sequence
  Heavy chain of chimeric antibody
MGWTLVFLFLLSVTAGVHSQVQLQQSGAELVRPGASVKLSCKALDYTFTDYEMHWVKQTPVHGLEWIGAIHPGRGGTAYNQKFKGKATLTADKSSSTAYMELSSLTSEDSGVYYCTSYHGGYWGQGTTLTVSSASTKGPSVFPLAPSSKSTSGGTAALGCLVKDYFPEPVTVSWNSGALTSGVHTFPAVLQSSGLYSLSSVVTVPSSSLGTQTYICNVNHKPSNTKVDKKVEPKSCDKTHTCPPCPAPELLGGPSVFLFPPKPKDTLMISRTPEVTCVVVDVSHEDPEVKFNWYVDGVEVHNAKTKPREEQYNSTYRVVSVLTVLHQDWLNGKEYKCKVSNKALPAPIEKTISKAKGQPREPQVYTLPPSRDELTKNQVSLTCLVKGFYPSDIAVEWESNGQPENNYKTTPPVLDSDGSFFLYSKLTVDKSRWQQGNVFSCSVMHEALHNHYTQKSLSLSPGK

SEQ ID NO: 42 - DNA, 1389 bp, Artificial Sequence
  Heavy chain of humanized antibody
atgggctggacgctcgtattcctctttcttctgtccgttacggcaggagtccactctcaggtgcagctggtccaatctggagctgaggtcaagaaaccaggcgctagcgtgatgttgagctgtaaagcctccgactacacatttaccgactacgagatgcactgggtgaaacaggctcctgtgcatggcctcgaatggattggcgcaatccatcccggaagaggaggtacagcctataaccagaagttcaaaggtcgggtgtccatgactcgagacacatctactagcacggtttatctggaactgagttctctgcgctctgaggatacagccgtgtattactgcaccagttaccatggcggctattggggtcaagggactttggtgacagtaagttccgcatccacaaagggtccatcagtctttccccttgcaccttcatccaagtccacatctggcgggacagctgccttggggtgcttggtcaaggactactttccagaaccagtgactgtcagttggaactctggagccctgacttctggagtgcataccttcccagccgtgctgcaatcaagcgggctgtacagtctgtccagtgtcgtgactgttccctcttcatccctcggtacccagacttacatctgcaatgtcaaccacaaacctagcaataccaaggtagacaagaaggtggagcccaaatcctgcgataagactcatacctgtcctccctgtcctgctcctgaacttcttggcggacccagtgtattcctgtttcctccaaagcccaaggacaccctcatgatcagcaggaccccagaagtgacctgtgtggtagtggacgtcagccacgaagatcccgaagtgaagttcaattggtacgttgatggcgtcgaggttcacaacgccaagaccaagcccagggaggaacagtacaattccacttatcgggttgtgtcagtgctgaccgttctgcatcaggattggcttaatggcaaggagtataagtgcaaggtttccaacaaagcactgccagctcctatcgagaaaaccattagcaaagccaaaggtcagccaagagagcctcaggtctatactctgcctccttctcgtgatgagctgaccaagaaccaggtcagcctgacatgtctcgtgaaagggttttaccccagcgacatagctgtggagtgggagtccaatgggcagcccgagaacaactacaagaccacaccacccgtgttggatagcgatggctccttctttctgtatagcaagctgacagttgacaagagtcgctggcaacaggggaatgtgttctcttgctcagtaatgcacgaagccctgcacaaccactatacccagaaatctctctccctgtcacccggaaaa

SEQ ID NO: 43 - protein, 463 aa, Artificial Sequence
  Heavy chain of humanized antibody
MGWTLVFLFLLSVTAGVHSQVQLVQSGAEVKKPGASVMLSCKASDYTFTDYEMHWVKQAPVHGLEWIGAIHPGRGGTAYNQKFKGRVSMTRDTSTSTVYLELSSLRSEDTAVYYCTSYHGGYWGQGTLVTVSSASTKGPSVFPLAPSSKSTSGGTAALGCLVKDYFPEPVTVSWNSGALTSGVHTFPAVLQSSGLYSLSSVVTVPSSSLGTQTYICNVNHKPSNTKVDKKVEPKSCDKTHTCPPCPAPELLGGPSVFLFPPKPKDTLMISRTPEVTCVVVDVSHEDPEVKFNWYVDGVEVHNAKTKPREEQYNSTYRVVSVLTVLHQDWLNGKEYKCKVSNKALPAPIEKTISKAKGQPREPQVYTLPPSRDELTKNQVSLTCLVKGFYPSDIAVEWESNGQPENNYKTTPPVLDSDGSFFLYSKLTVDKSRWQQGNVFSCSVMHEALHNHYTQKSLSLSPGK

SEQ ID NO: 44 - DNA, 1389 bp, Artificial Sequence
  Heavy chain of humanized antibody
atggggtggacacttgtctttctctttctgctgtctgttaccgctggcgtacactcccaagtacagctggtccaaagcggcgctgaagtcgtgcgacccggggcaagcgtgaaactgtcctgtaaagcctccgactatactttcactgattacgagatgcattgggtacgacaggcaccaggccagggtcttgagtgggttggcgctattcatcctggtcggggtggaaccgcctacaatcagaagttcaaaggccgcgtgacaattactgccgataagtcaacaagtaccgcttacatggaattgtcatccctgcgcagtgaggatactgccgtctactattgcacctcctatcatggaggatattggggccaagggactaccgtgaccgtaagttctgcctcaacaaaagggccctctgtgtttcccctggcaccctctagcaagagtacaagcggaggcacagctgccctgggttgtctggtgaaagactactttcctgagccagtcacagtgtcatggaatagcggagcactgacttctggagtgcacacctttcccgcagtcttgcagagttctggcctgtattccctctcctccgttgttacagtcccatcctcttctctcgggacccagacatacatctgcaacgtgaaccacaagcctagcaacacgaaggtggacaagaaagttgagcccaagagctgtgataagacccacacttgcccaccttgtccagcccctgaactccttggtggtccaagcgtgttcctctttccaccaaagcctaaggacaccttgatgatcagcaggactcctgaagtgacgtgtgtggtggtggacgtgtcccatgaagatcccgaggtcaagttcaattggtatgtagacggggtagaggttcacaacgctaaaacaaaaccccgtgaggagcagtacaacagcacatatcgggtcgtcagtgtccttaccgtgctgcatcaggattggctgaatggaaaggagtataagtgcaaagtgtccaacaaggccctgcccgctcccatcgagaaaaccatctctaaggctaaaggccagcccagagaacctcaggtgtataccctcccaccttcaagggacgaattgaccaagaatcaggtgtcccttacttgcttggttaaaggcttctacccctcagacatagccgttgagtgggaatcaaatggacagcctgagaacaactacaaaaccacgcctccagtgctggattccgatggctccttctttctgtactctaagctgacagtcgacaagagtagatggcagcaagggaatgtgttcagctgcagtgttatgcatgaagccctgcacaaccactacactcagaagtctctgagcctgtctcccggtaag

SEQ ID NO: 45 - protein, 463 aa, Artificial Sequence
  Heavy chain of humanized antibody
MGWTLVFLFLLSVTAGVHSQVQLVQSGAEVVRPGASVKLSCKASDYTFTDYEMHWVRQAPGQGLEWVGAIHPGRGGTAYNQKFKGRVTITADKSTSTAYMELSSLRSEDTAVYYCTSYHGGYWGQGTTVTVSSASTKGPSVFPLAPSSKSTSGGTAALGCLVKDYFPEPVTVSWNSGALTSGVHTFPAVLQSSGLYSLSSVVTVPSSSLGTQTYICNVNHKPSNTKVDKKVEPKSCDKTHTCPPCPAPELLGGPSVFLFPPKPKDTLMISRTPEVTCVVVDVSHEDPEVKFNWYVDGVEVHNAKTKPREEQYNSTYRVVSVLTVLHQDWLNGKEYKCKVSNKALPAPIEKTISKAKGQPREPQVYTLPPSRDELTKNQVSLTCLVKGFYPSDIAVEWESNGQPENNYKTTPPVLDSDGSFFLYSKLTVDKSRWQQGNVFSCSVMHEALHNHYTQKSLSLSPGK

SEQ ID NO: 46 - DNA, 1389 bp, Artificial Sequence
  Heavy chian of humanized antibody
atgggctggacactggtgtttctctttctccttagcgttaccgccggtgtgcactctcaggttcagctggtgcagtcaggagctgaggtgaagaaaccaggcgcttctgtgaaggtgtcttgtaaagcctctgactacactttcaccgactatgagatgcattgggtccggcagacacccggacatggccttgaatggatgggagccattcatcctggcagaggagggacagcctataaccagaagttcaagggacgcgttactatgaccgctgacaagtccatttccaccgcctacatggagctcaactcactgacttctgacgattcagccgtgtactactgtaccagctatcacggcgggtattggggacaggggaccctggtgactgtgtctagtgcaagcacaaaaggaccctctgttttccctctggctccttcctctaagagcacttcaggtggcaccgcagccttgggttgtctggtgaaggactactttccagaacctgtgacagtctcatggaactctggtgctctgacaagcggcgtgcatacttttccagctgtcctgcagagttccggcctgtattctctgtcctcagtcgtcactgtgccctctagttccttggggacccaaacctacatctgcaatgtcaatcacaaacctagtaatacgaaagtagacaagaaagtagagcccaagagctgcgacaagacccacacatgccctccatgtccagcacctgaattgctgggtggcccatccgtgtttctgtttcctcccaaaccaaaagatacactgatgatcagccggactcccgaagtgacctgtgtagttgtggacgtcagccatgaagatcccgaggtcaaattcaactggtatgttgatggtgtagaggttcacaatgccaagactaagccacgagaggaacagtacaatagcacctatcgtgtcgtaagtgtccttaccgtcctccaccaagactggcttaacggcaaagagtacaagtgcaaagtctctaacaaggcactccctgcaccaatcgagaaaacgatcagcaaggccaaggggcaacccagagaaccccaggtttatactctgccaccctccagggatgagttgacgaagaatcaggtgtccctgacatgcctcgtgaaagggttctaccccagtgatatagccgtagaatgggagtccaatggtcagcccgagaacaactacaagacaacacctcccgtgctggatagcgacggaagtttcttcctgtactccaagttgaccgtggataagtccaggtggcaacaggggaatgtgtttagctgctcagtgatgcacgaagctcttcacaaccattatacccagaaatccctgtccctgagtcctggcaag

SEQ ID NO: 47 - protein, 463 aa, Artificial Sequence
  Heavy chain of humanized antibody
MGWTLVFLFLLSVTAGVHSQVQLVQSGAEVKKPGASVKVSCKASDYTFTDYEMHWVRQTPGHGLEWMGAIHPGRGGTAYNQKFKGRVTMTADKSISTAYMELNSLTSDDSAVYYCTSYHGGYWGQGTLVTVSSASTKGPSVFPLAPSSKSTSGGTAALGCLVKDYFPEPVTVSWNSGALTSGVHTFPAVLQSSGLYSLSSVVTVPSSSLGTQTYICNVNHKPSNTKVDKKVEPKSCDKTHTCPPCPAPELLGGPSVFLFPPKPKDTLMISRTPEVTCVVVDVSHEDPEVKFNWYVDGVEVHNAKTKPREEQYNSTYRVVSVLTVLHQDWLNGKEYKCKVSNKALPAPIEKTISKAKGQPREPQVYTLPPSRDELTKNQVSLTCLVKGFYPSDIAVEWESNGQPENNYKTTPPVLDSDGSFFLYSKLTVDKSRWQQGNVFSCSVMHEALHNHYTQKSLSLSPGK

SEQ ID NO: 48 - DNA, 1389 bp, Artificial Sequence
  Heavy chain of humanized antibody
atgggttggactcttgttttcttgttcctgttgagtgtgactgccggagtacactctcaggtgcaactccaacagagcggcgctgaggtggttcgaccaggcgcatccgtgaaggtgtcatgcaaagctagcgactacacctttaccgactatgagatgcattgggttaagcaggctcctggacaagggctggagtggataggcgctattcatcctggcaggggtggaaccgcatataaccagaagttcaaaggcagagtgacgatgacagccgataccagcatcagcacagcctatatggagctgtccagacttcgatccgacgataccgccgtctattactgcactagttatcacggcggttattggggtcagggtacaactctgacagtaagttctgcctctacgaaaggtccctccgtctttcccctcgcaccttcttccaagagcacaagtggaggaacagcagccctggggtgtttggtgaaggactacttcccagaacctgtgaccgtgagttggaattctggtgccctgacatccggggtccatacctttcccgcagtgcttcagtccagtggactctactctctgtctagcgttgtcaccgtgccctcatctagcctgggcacacagacctacatctgtaacgtgaatcacaaaccctccaacactaaagtcgacaagaaagtggaacctaagagctgcgataagacccatacatgcccaccatgtcctgctcctgaacttcttggcgggccatcagtgtttctgttccctccaaaacccaaggacaccctcatgattagcaggacaccagaagtcacctgtgtggtggtcgacgtatctcacgaggatccagaggtgaaatttaactggtatgtagacggcgttgaggtgcataatgccaagactaaaccccgggaagaacagtacaactccacctatcgcgtagtctcagttctgactgtgctgcaccaggattggttgaacgggaaggagtacaagtgtaaagtcagtaacaaagctctgccagctcccatcgaaaagaccatctcaaaggccaaggggcagcctcgtgaaccccaggtctacactctcccacccagccgggatgaactgacgaagaatcaggtatcactgacatgcctggtcaaaggcttttatcccagtgacattgccgtggagtgggagtccaatggacaacctgagaacaactacaagacaactcctcccgttctggatagcgatgggtccttcttcctgtacagcaagctcactgttgacaaatcacgctggcagcagggaaatgtgttttcctgctctgtgatgcatgaggctctgcacaatcactacacccagaagtccctgtccttgtctcccggcaag

SEQ ID NO: 49 - protein, 463 aa, Artificial Sequence
  Heavy chain of humanized antibody
MGWTLVFLFLLSVTAGVHSQVQLQQSGAEVVRPGASVKVSCKASDYTFTDYEMHWVKQAPGQGLEWIGAIHPGRGGTAYNQKFKGRVTMTADTSISTAYMELSRLRSDDTAVYYCTSYHGGYWGQGTTLTVSSASTKGPSVFPLAPSSKSTSGGTAALGCLVKDYFPEPVTVSWNSGALTSGVHTFPAVLQSSGLYSLSSVVTVPSSSLGTQTYICNVNHKPSNTKVDKKVEPKSCDKTHTCPPCPAPELLGGPSVFLFPPKPKDTLMISRTPEVTCVVVDVSHEDPEVKFNWYVDGVEVHNAKTKPREEQYNSTYRVVSVLTVLHQDWLNGKEYKCKVSNKALPAPIEKTISKAKGQPREPQVYTLPPSRDELTKNQVSLTCLVKGFYPSDIAVEWESNGQPENNYKTTPPVLDSDGSFFLYSKLTVDKSRWQQGNVFSCSVMHEALHNHYTQKSLSLSPGK

SEQ ID NO: 50 - DNA, 1389 bp, Artificial Sequence
  Heavy chain of humanized antibody
atgggatggacactggtgtttctgttccttctcagtgtgacagctggggtccattcccaagtgcaactgcagcaatcaggcgctgaagttaagcggccaggtgctagcgtaaaagtctcttgcaaggcatccgactacacatttaccgactatgagatgcactgggtgcgtcagacacctgggcatggtctggagtggatgggagccattcacccaggaagaggaggcactgcctacaatcagaagttcaaaggaagggttaccatgaccgctgataagtctacatctaccgtctacatggagctgagttccctgacttccgaggatactgccgtgtactactgcacatcctaccacggcggatattggggccaggggaccaccttgacagtctcctccgcttctaccaagggcccatctgtgtttcctctggccccatccagcaaaagtacttcaggtggcaccgctgcattgggctgtctggtgaaggactattttcctgaacccgtgacggtttcctggaattccggtgcactgacatccggggtgcatacatttcccgctgttctgcagagttctgggctttacagcctgagctctgtggtcactgtacccagtagctcattggggacccagacctatatctgcaatgtcaatcacaaaccctccaatacaaaagtcgacaagaaggtggaaccaaagtcatgtgacaagacgcatacttgcccaccctgtcccgcacccgaactgcttggtggcccttccgtattcctctttccacccaagcctaaagacaccttgatgatctctaggaccccagaagtgacttgcgtcgtagtggatgtatcccacgaagatccagaggtgaagttcaactggtatgtggacggtgttgaggtccacaacgccaaaactaagcctcgcgaagagcagtataacagcacctatcgggtcgtttctgtgctcacagttctgcatcaggactggctgaatggcaaggagtacaagtgtaaagtgagcaacaaagcccttcctgcccctattgagaaaacaatcagcaaggcaaagggccaacccagagagccccaggtctacactctgcctccctcacgcgacgagctcactaagaaccaggtttcactgacttgtctcgtgaagggtttctatcccagcgatatagccgtggaatgggagtctaatggacagcccgaaaacaactacaagaccaccccacctgtattggatagcgatggaagtttcttcctgtattctaagctgacggtggataaaagccgatggcagcaggggaacgtgtttagctgctctgtgatgcatgaggccctccacaaccactacacccagaaatcacttagtctgagtcctggcaaa

SEQ ID NO: 51 - protein, 463 aa, Artificial Sequence
  Heavy chain of humanized antibody
MGWTLVFLFLLSVTAGVHSQVQLQQSGAEVKRPGASVKVSCKASDYTFTDYEMHWVRQTPGHGLEWMGAIHPGRGGTAYNQKFKGRVTMTADKSTSTVYMELSSLTSEDTAVYYCTSYHGGYWGQGTTLTVSSASTKGPSVFPLAPSSKSTSGGTAALGCLVKDYFPEPVTVSWNSGALTSGVHTFPAVLQSSGLYSLSSVVTVPSSSLGTQTYICNVNHKPSNTKVDKKVEPKSCDKTHTCPPCPAPELLGGPSVFLFPPKPKDTLMISRTPEVTCVVVDVSHEDPEVKFNWYVDGVEVHNAKTKPREEQYNSTYRVVSVLTVLHQDWLNGKEYKCKVSNKALPAPIEKTISKAKGQPREPQVYTLPPSRDELTKNQVSLTCLVKGFYPSDIAVEWESNGQPENNYKTTPPVLDSDGSFFLYSKLTVDKSRWQQGNVFSCSVMHEALHNHYTQKSLSLSPGK

SEQ ID NO: 52 - DNA, 717 bp, Artificial Sequence
  Light chain of chimeric antibody
atggttagctccgctcagtttctgggacttctgctgttgtgctttcaagggactcggtgtgatgttgtcatgacgcaaacacccctgtcactgcctgtgtcactgggagatcaggcctccattagttgcagaagttctcagtccttggtgcactcaaatgagaacacctaccttctgtggtatctgcagaaaccaggccagtctcccaagctcctgatctacaaggtgtctaatcgcttcagtggcgttcctgacaggtttagtgggtccggttcagggaccgatttcaccctcaagataagccgagtagaggcagaggatcttggcgtttacttctgcagtcagacaactcatgtgccatggacttttggcggtggcaccaaactggagattaagcgtacagtggcagctccatctgtgttcatctttcctcccagcgatgagcagctgaaatccgggacagcttccgtcgtgtgtttgctcaacaacttctatcccagggaagccaaggtacagtggaaggtcgacaatgccctccagtcaggaaactcccaagagagcgtgaccgaacaggactccaaagactccacctatagcttgtctagcactctcactctgtctaaagccgactacgagaagcacaaggtgtatgcctgtgaagtcacccatcagggactgtctagccctgtcacaaagagcttcaatcggggtgaatgc

SEQ ID NO: 53 - protein, 239 aa, Artificial Sequence
  Light chain of chimeric antibody
MVSSAQFLGLLLLCFQGTRCDVVMTQTPLSLPVSLGDQASISCRSSQSLVHSNENTYLLWYLQKPGQSPKLLIYKVSNRFSGVPDRFSGSGSGTDFTLKISRVEAEDLGVYFCSQTTHVPWTFGGGTKLEIKRTVAAPSVFIFPPSDEQLKSGTASVVCLLNNFYPREAKVQWKVDNALQSGNSQESVTEQDSKDSTYSLSSTLTLSKADYEKHKVYACEVTHQGLSSPVTKSFNRGEC

SEQ ID NO: 54 - DNA, 717 bp, Artificial Sequence
  Light chain of humanized antibody
atggtgagctctgcccagtttctgggcctgttgctcctgtgctttcagggtacacgatgtgacatcgtgatgacgcagactcctctgtctagtcccgtgactcttggccagcctgcatccattagttgcaggagttctcagagcctggtccatagcaacgagaacacctatctgctctggtatctgcaaagacccggtcaaccacccaaactgctcatctacaaggtgtccaatcgcttttctggggttccagacaggttctcaggatccggtgcaggaaccgatttcacgctgaagattagccgtgtagaagccgaggatgtaggcgtgtacttctgctcccagactacccatgttccctggacatttgggcagggaaccaagttggagataaaacggactgtcgcagctccttccgtgttcatctttcctccctctgatgagcagctgaaatccgggacagcttccgtggtttgcttgctcaacaacttctatccaagagaagccaaagtccagtggaaggtcgacaatgctctgcagtcaggcaattcacaggagtctgtgacagagcaagactccaaggatagtacctactcccttagctctacccttaccctgagtaaagccgactacgaaaagcacaaggtctatgcctgtgaagtgacacaccaaggcctgtcaagcccagttactaagagcttcaatcggggagagtgt

SEQ ID NO: 55 - protein, 239 aa, Artificial Sequence
  Light chain of humanized antibody
MVSSAQFLGLLLLCFQGTRCDIVMTQTPLSSPVTLGQPASISCRSSQSLVHSNENTYLLWYLQRPGQPPKLLIYKVSNRFSGVPDRFSGSGAGTDFTLKISRVEAEDVGVYFCSQTTHVPWTFGQGTKLEIKRTVAAPSVFIFPPSDEQLKSGTASVVCLLNNFYPREAKVQWKVDNALQSGNSQESVTEQDSKDSTYSLSSTLTLSKADYEKHKVYACEVTHQGLSSPVTKSFNRGEC

SEQ ID NO: 56 - DNA, 717 bp, Artificial Sequence
  Light chain of humanized antibody
atggtcagctcagcccagtttctgggactcctcttgctgtgctttcagggcactcgttgcgacatagtcatgacacaatcaccactgtccctttctgtgacacctggacagccagcttccatttcctgccggtctagtcagtctctggtccatagcaacgagaacacctatcttctgtggtatctccagaagcctgggcaatctccccagttgctcatctacaaggtgtccaataggttctcaggtgttcccgatcgctttagcggatctgggtcaggtaccgacttcaccctgaagatcagtagggtggaagccgaggatgtgggcgtgtacttctgttcccagacaacacacgtaccctggacgtttggacaagggaccaaagtggagattaagcggaccgttgcagctcctagtgtgtttatcttccctccatctgatgagcagctgaagagcggcactgctagtgtagtctgtctgctgaacaacttctatcccagagaagccaaagtccagtggaaggtggacaatgccctgcaatccggcaatagccaggagagcgttaccgaacaggactctaaggatagcacatactccctttcctccactctgactctgtctaaagccgactacgagaaacacaaagtgtatgcatgtgaggtgactcatcagggtttgagtagccccgttaccaagtcattcaatcgaggcgaatgc

SEQ ID NO: 57 - protein, 239 aa, Artificial Sequence
  Light chain of humanized antibody
MVSSAQFLGLLLLCFQGTRCDIVMTQSPLSLSVTPGQPASISCRSSQSLVHSNENTYLLWYLQKPGQSPQLLIYKVSNRFSGVPDRFSGSGSGTDFTLKISRVEAEDVGVYFCSQTTHVPWTFGQGTKVEIKRTVAAPSVFIFPPSDEQLKSGTASVVCLLNNFYPREAKVQWKVDNALQSGNSQESVTEQDSKDSTYSLSSTLTLSKADYEKHKVYACEVTHQGLSSPVTKSFNRGEC

SEQ ID NO: 58 - DNA, 717 bp, Artificial Sequence
  Light chain of humanized antibody
atggtcagttctgcccaattccttgggctgcttctgctctgctttcagggcacaagatgcgacattcagatgacccagtcaccttcctctctgtccgctagtgtgggagatagggtcaccattacatgtcgctcatcccagtcactggttcacagcaatgagaacacctacctgttgtggtatctgcagaaacccggtcaagcacccaaactgctgatctacaaggtgtctaatcggttctcaggagtaccatcccggtttagcggaagtgggtctggcactgactttaccctgaccatctcttcactgcaacctgaggatttcgccacctacttttgctcccagacgactcatgtgccttggacatttggtggcggtaccaagctcgagataaagcgtaccgttgctgctccctccgtgttcatctttccaccttccgatgaacagctgaagtccggaactgcatctgtcgtgtgtttgctgaacaacttctatcccagggaagccaaagtgcagtggaaggttgacaacgcactgcagtctggcaattcccaggagagtgtaacagagcaggatagcaaagacagcacgtactctttgtccagcacactcactctcagcaaagccgactatgagaagcacaaggtgtatgcctgtgaagtcacacatcaagggcttagcagtccagtgactaagagcttcaatcgaggcgaatgc

SEQ ID NO: 59 - protein, 239 aa, Artificial Sequence
  Light chain of humanized antibody
MVSSAQFLGLLLLCFQGTRCDIQMTQSPSSLSASVGDRVTITCRSSQSLVHSNENTYLLWYLQKPGQAPKLLIYKVSNRFSGVPSRFSGSGSGTDFTLTISSLQPEDFATYFCSQTTHVPWTFGGGTKLEIKRTVAAPSVFIFPPSDEQLKSGTASVVCLLNNFYPREAKVQWKVDNALQSGNSQESVTEQDSKDSTYSLSSTLTLSKADYEKHKVYACEVTHQGLSSPVTKSFNRGEC